European Patent Specification EP 2 841 452 B1, published April 12, 2023. Title: MODIFIED GLYCOPROTEINS. Applicant: Meador, James  III Bosques, Carlos J. Bulik, Dorota A. Bhatnagar, Naveen Brown, Julia Markowitz, Lynn Prabbhakar, Sathya. Application PCT/US13/37997. The sequence listing filed with the application follows.

SEQUENCE LISTING (5 sequences)

SEQ ID NO: 1 - protein, 470 aa, Homo sapiens
MGWSLILLFLVAVATRVLSQVQLQQPGAELVKPGASVKMSCKASGYTFTSYNMHWVKQTPGRGLEWIGAIYPGNGDTSYNQKFKGKATLTADKSSSTAYMQLSSLTSEDSAVYYCARSTYYGGDWYFNVWGAGTTVTVSAASTKGPSVFPLAPSSKSTSGGTAALGCLVKDYFPEPVTVSWNSGALTSGVHTFPAVLQSSGLYSLSSVVTVPSSSLGTQTYICNVNHKPSNTKVDKKAEPKSCDKTHTCPPCPAPELLGGPSVFLFPPKPKDTLMISRTPEVTCVVVDVSHEDPEVKFNWYVDGVEVHNAKTKPREEQYNSTYRVVSVLTVLHQDWLNGKEYKCKVSNKALPAPIEKTISKAKGQPREPQVYTLPPSRDELTKNQVSLTCLVKGFYPSDIAVEWESNGQPENNYKTTPPVLDSDGSFFLYSKLTVDKSRWQQGNVFSCSVMHEALHNHYTQKSLSLSPGK

SEQ ID NO: 2 - protein, 470 aa, Homo sapiens
  MISC_FEATURE (264)..(264): F241A
  MISC_FEATURE (266)..(266): F243A
MGWSLILLFLVAVATRVLSQVQLQQPGAELVKPGASVKMSCKASGYTFTSYNMHWVKQTPGRGLEWIGAIYPGNGDTSYNQKFKGKATLTADKSSSTAYMQLSSLTSEDSAVYYCARSTYYGGDWYFNVWGAGTTVTVSAASTKGPSVFPLAPSSKSTSGGTAALGCLVKDYFPEPVTVSWNSGALTSGVHTFPAVLQSSGLYSLSSVVTVPSSSLGTQTYICNVNHKPSNTKVDKKAEPKSCDKTHTCPPCPAPELLGGPSVALAPPKPKDTLMISRTPEVTCVVVDVSHEDPEVKFNWYVDGVEVHNAKTKPREEQYNSTYRVVSVLTVLHQDWLNGKEYKCKVSNKALPAPIEKTISKAKGQPREPQVYTLPPSRDELTKNQVSLTCLVKGFYPSDIAVEWESNGQPENNYKTTPPVLDSDGSFFLYSKLTVDKSRWQQGNVFSCSVMHEALHNHYTQKSLSLSPGK

SEQ ID NO: 3 - protein, 470 aa, Homo sapiens
  MISC_FEATURE (266)..(266): F243A
  MISC_FEATURE (324)..(324): R301A
MGWSLILLFLVAVATRVLSQVQLQQPGAELVKPGASVKMSCKASGYTFTSYNMHWVKQTPGRGLEWIGAIYPGNGDTSYNQKFKGKATLTADKSSSTAYMQLSSLTSEDSAVYYCARSTYYGGDWYFNVWGAGTTVTVSAASTKGPSVFPLAPSSKSTSGGTAALGCLVKDYFPEPVTVSWNSGALTSGVHTFPAVLQSSGLYSLSSVVTVPSSSLGTQTYICNVNHKPSNTKVDKKAEPKSCDKTHTCPPCPAPELLGGPSVFLAPPKPKDTLMISRTPEVTCVVVDVSHEDPEVKFNWYVDGVEVHNAKTKPREEQYNSTYAVVSVLTVLHQDWLNGKEYKCKVSNKALPAPIEKTISKAKGQPREPQVYTLPPSRDELTKNQVSLTCLVKGFYPSDIAVEWESNGQPENNYKTTPPVLDSDGSFFLYSKLTVDKSRWQQGNVFSCSVMHEALHNHYTQKSLSLSPGK

SEQ ID NO: 4 - protein, 470 aa, Homo sapiens
  MISC_FEATURE (269)..(269): K246A
  MISC_FEATURE (283)..(283): T260A
MGWSLILLFLVAVATRVLSQVQLQQPGAELVKPGASVKMSCKASGYTFTSYNMHWVKQTPGRGLEWIGAIYPGNGDTSYNQKFKGKATLTADKSSSTAYMQLSSLTSEDSAVYYCARSTYYGGDWYFNVWGAGTTVTVSAASTKGPSVFPLAPSSKSTSGGTAALGCLVKDYFPEPVTVSWNSGALTSGVHTFPAVLQSSGLYSLSSVVTVPSSSLGTQTYICNVNHKPSNTKVDKKAEPKSCDKTHTCPPCPAPELLGGPSVFLFPPAPKDTLMISRTPEVACVVVDVSHEDPEVKFNWYVDGVEVHNAKTKPREEQYNSTYRVVSVLTVLHQDWLNGKEYKCKVSNKALPAPIEKTISKAKGQPREPQVYTLPPSRDELTKNQVSLTCLVKGFYPSDIAVEWESNGQPENNYKTTPPVLDSDGSFFLYSKLTVDKSRWQQGNVFSCSVMHEALHNHYTQKSLSLSPGK

SEQ ID NO: 5 - protein, 470 aa, Homo sapiens
  MISC_FEATURE (283)..(283): T260A
  MISC_FEATURE (324)..(324): R301A
MGWSLILLFLVAVATRVLSQVQLQQPGAELVKPGASVKMSCKASGYTFTSYNMHWVKQTPGRGLEWIGAIYPGNGDTSYNQKFKGKATLTADKSSSTAYMQLSSLTSEDSAVYYCARSTYYGGDWYFNVWGAGTTVTVSAASTKGPSVFPLAPSSKSTSGGTAALGCLVKDYFPEPVTVSWNSGALTSGVHTFPAVLQSSGLYSLSSVVTVPSSSLGTQTYICNVNHKPSNTKVDKKAEPKSCDKTHTCPPCPAPELLGGPSVFLFPPKPKDTLMISRTPEVACVVVDVSHEDPEVKFNWYVDGVEVHNAKTKPREEQYNSTYAVVSVLTVLHQDWLNGKEYKCKVSNKALPAPIEKTISKAKGQPREPQVYTLPPSRDELTKNQVSLTCLVKGFYPSDIAVEWESNGQPENNYKTTPPVLDSDGSFFLYSKLTVDKSRWQQGNVFSCSVMHEALHNHYTQKSLSLSPGK